European Patent Specification EP 3 912 630 B1, published October 11, 2023. Title: METHODS AND COMPOSITIONS FOR CHANGING THE COMPOSITION OF THE SKIN MICROBIOME USING COMPLEX MIXTURES OF BACTERIAL STRAINS. Applicant: Patzold, Bernhard Guell, Marc. Application Not Yet Assigned. The sequence listing filed with the application follows.

SEQUENCE LISTING (82 sequences)

SEQ ID NO: 1 - DNA, 484 bp, Propionibacterium acnes
gttgcacaccagggggtcaacttggcgtcctcagttcaaaattgattcaaactaacagttccatgtcgggaaacagcaccaggaagctcgtgacatatcgtctttcattgcgagaaacatcttacttatgtacatttctaagctatagcgtctacccttgtcagacccaggacgatgggtgtcacatctcctttctagtcaacctaagagaggaggaaatgccgcgatatatgttccaccctgtcatcacgaaggccaccacaatctatcccagaacagccggcacttcactcacgatgccccgatgctggattcctattgtcgcccttattagggcaagcggtgccagtagcagaatatgtcacctcaacaactcgatccacccctgcccattacatgggtaacatatccatggaggttcgatgtatactcgaggatacagtcgtccatcacgcccgcctacatacccattacatcagcatag

SEQ ID NO: 2 - DNA, 484 bp, Propionibacterium acnes
gttgcacaccagggggtcaacttggcgtcctcagttcaaaattgattcaaactaacagttccatgtcgggaaacagcaccaggaagctcgtgacatatcgtctttcattgcgagaaacatcttacttatgtacatttctaagctatagcgtctacccttgtcagacccaggacgatgggtgtcacatctcctttctagtcaacctaagagaggaggaaatgccgcgatatatgttccaccctgtcatcacgaaggccaccacaatctatcccagaacagccggcacttcactcacgatgccccgattctggattcctattgtcgcccttattagggcaagcggtgccagtagcagaatatgtcacctcaacaactcgatccacccctgcccattacatgggtaacatatccatggaggttcgatgtatactcgaggatacagtcgtccatcacgcccgcctacatacccattacatcagcatag

SEQ ID NO: 3 - DNA, 484 bp, Propionibacterium acnes
gttgcacaccagggggtcaacttggcgtcctcagttcaaaattgattcaaactaacagttccatgtcgggaaacagcaccaggaagctcgtgacatatggtctttcattgcgagaaacatcttacttatgtacatttctaagctatagcgtctacccttgtcagacccaggacgatgggtgtcacatctcctttctagtcaacctaagagaggaggaaatgccgcgatatatgttccaccctgtcatcacgaaggccaccacaatctatcccagaacagccggcacttcactcacgatgccccgatgctggattcctattgtcgcccttattagggcaagcggtgccagtagcagaatatgtcacctcaataactcgatccacccctgcccattacatgggtaacatatccatggaggttcgatgtatactcgaggatacagtcgtccatcacgcccgcctacatacccattacatcagcatag

SEQ ID NO: 4 - DNA, 484 bp, Propionibacterium acnes
gttgcacaccagggggtcaacttggcgtcctcagttcaaaattgattcaaactaacagttccatgtcgggaaacagcaccaggaagctcgtgacatatggtctttcattgcgagaaacatcttacttatgtacatttctaagctatagcgtctacccttgtcagacccaggacgatgggtgtcacatctcctttctagtcaacctaagagaggaggaaatgccgcgatatatgttccaccctgtcatcacgaaggccaccacaatctatcccagaacagccggcacttcactcacgatgccccgatgctggattcctattgtcgcccttattagggcaagcggtgccagtagcagaatatgtcacctcaacaactcgatccacccctgcccattacatgggtaacatatccatggaggttcgatgtatactcgaggatacagtcgtccatcacgcccgcctacatacccattacatcagcatag

SEQ ID NO: 5 - DNA, 484 bp, Propionibacterium acnes
gttgcacaccagggggtcaacttggcgtcctcagttcaaaattgattcaaactaacagttccatgccgggaaacagcaccaggaagctcgtgacatatcgtctttcattgcgagaaacatcttacttatgtacatttctaagctatagcgtctacccttgtcagacccaggacgatgggtgtcacatctcctttctagtcaacctaagagaggaggaaatgccgcgatatatgttccaccctgtcatcacgaaggccaccacaatctatcccagaacagccggcacttcactcacgatgccccgatgctggattcctattgtcgcccttattagggcaagcggtgccagtagcagaatatgtcacctcaacaactcgatccacccctgcccattacatgggtaacatatccatggaggttcgatgtatactcgaggatacagtcgtccatcacgcccgcctacatacccattacatcagcatag

SEQ ID NO: 6 - DNA, 484 bp, Propionibacterium acnes
gttgcacaccagggggtcaacttggcgtcctcagttcaaaattgattcaaactaacagttccatgtcgggaaacagcaccaggaagctcgtgacatatcgtctttcattgcgagaaacatcttacttatgtacatttctaagctatagcgtctacccttgtcagacccaggacgatgggtgtcacatctcctttctagtcaacctaagagaggaggaaatgccgcgatatatgttccaccctgtcatcacgaaggccaccacaatctatcccagaacagccggcacttcactcacgatgccccgatgctggattcctattgtcgcccttattagggcaagcggtgccagtagcagaatatgtcacctcaacaactcgatccacccctgcccattacatgggtaacatatccatggaggttcgatgtatactcgaggatacagtcgtccatcacgcccgcctacatacccattacatcagcatat

SEQ ID NO: 7 - DNA, 484 bp, Propionibacterium acnes
gttgcacaccagggggtcaacttggcgtcctcagttcaaaattgattcaaactaacagttccatgtcgggaaacagcaccaggaagctcgtgacatatcgtctttcattgcgagaaacatcttacttatgtacatttctaagctatagcgtctacccttgtcagacccaggacgatgggtgtcacatctcctttctagtcaacctaagagaggaggaaatgccgcgatatatgttccaccctgccatcacgaaggccaccacaatctatcccagaacagccggcacttcactcacgatgccccgattctggattcctattgtcgcccttattagggcaagcggtgccagtagcagaatatgtcacctcaacaactcgatccacccctgcccattacatgggtaacatatccatggaggttcgatgtatactcgaggatacagtcgtccatcacgcccgcctacatacccattacatcagcatag

SEQ ID NO: 8 - DNA, 484 bp, Propionibacterium acnes
gttgcacaccagggggtcaacttggcgtcctcagttcaaaattgattcaaactaacagttccatgtcgggaaacagcaccaggaagctcgtgacatatcgcctttcattgcgagaaacatcttacttatgtacatttctaagctatagcgtctacccttgtcagacccaggacgatgggtgtcacatctcctttctagtcaacctaagagaggaggaaatgccgcgatatatgttccaccctgtcatcacgaaggccaccacaatctatcccagaacagccggcacttcactcacgatgccccgatgctggattcctattgtcgcccttattagggcaagcggtgccagtagcagaatatgtcacctcaacaactcgatccacccctgcccattacatgggtaacatatccatggaggttcgatgtatactcgaggatacagtcgtccatcacgcccgcctacatacccattacatcagcatag

SEQ ID NO: 9 - DNA, 484 bp, Propionibacterium acnes
gttgcacaccagggggtcaacttggcgtcctcagttcaaaattgattcaaactaacagttccatgccgggaaacagcaccaggaagctcgtgacatatcgtctttcattgcgagaaacatcttacttatgtacatttctaagctatagcgtctacccttgtcagacccaggacgatgggtgtcacatctcctttctagtcaacctaagagaggaggaaatgccgcgatatatgttccaccctgtcatcatgaaggccaccacaatctatcccagaacagccggcacttcactcacgatgccccgatgctggattcctattgtcgcccttattagggcaagcggtgccagtagcagaatatgtcacctcaacaactcgatccacccctgcccattacatgggtaacatatccatggaggttcgatgtatactcgaggatacagtcgtccatcacgcccgcctacatacccattacatcagcatag

SEQ ID NO: 10 - DNA, 484 bp, Propionibacterium acnes
gttgcacaccagggggtcaacttggcgtcctcagttcaaaattgattcaaactaacagttccatgccgggaaacagcaccaggaagctcgtgacatatcgtctttcattgcgagaaacatcttacttatgtacatttctaagctatagcgtctacccttgtcagacccaggacgatgggtgtcacatctcctttctagtcaacctaagagaggaggaaatgccgcgatatatgttccaccctgtcatcacgaaggccaccacaatctatcccagaacagccggcacttcactcacgatgccccgatgctggattcctattgtcgcccttattagggcaagcggtgccagtagcagaatatgtcacctcaacaactcgatctacccctgcccattacatgggtaacatatccatggaggttcgatgtatactcgaggatacagtcgtccatcacgcccgcctacatacccattacatcagcatag

SEQ ID NO: 11 - DNA, 484 bp, Propionibacterium acnes
gttgcacaccagggggtcaacttggcgtcctcagttcaaaattgattcaaactaacagttccatgccgggaaacagcaccaggaagcccgtgacatatcgtctttcattgcgagaaacatcttacttatgtacatttctaagctatagcgtctacccttgtcagacccaggacgatgggtgtcacatctcctttctagtcaacctaagagaggaggaaatgccgcgatatatgttccaccctgtcatcacgaaggccaccacaatctatcccagaacagccggcacttcactcacgatgccccgatgctggattcctattgtcgcccttattagggcaagcggtgccagtagcagaatatgtcacctcaacaactcgatccacccctgcccattacatgggtaacatatccatggaggttcgatgtatactcgaggatacagtcgtccatcacgcccgcctacatacccattacatcagcatag

SEQ ID NO: 12 - DNA, 484 bp, Propionibacterium acnes
gttgcacaccagggggtcaacttggcgtcctcagttcaaaattgattcaaactaacagttccatgccgggaaacagcaccaggaagctcgtgacatatcgtctttcattgcgagaaacatcttacttatgtacatttctaagctatagcgtctacccttgtcagacccaggacgatgggtgtcacatctcctttctagtcaacctaagagaggaggaaatgccgcgatatatattccaccctgtcatcacgaaggccaccacaatctatcccagaacagccggcacttcactcacgatgccccgatgctggattcctattgtcgcccttattagggcaagcggtgccagtagcagaatatgtcacctcaacaactcgatccacccctgcccattacatgggtaacatatccatggaggttcgatgtatactcgaggatacagtcgtccatcacgcccgcctacatacccattacatcagcatag

SEQ ID NO: 13 - DNA, 484 bp, Propionibacterium acnes
gttgcacaccagggggtcaacttggcgtcctcagttcaaaattgattcaaactaacagttccatgtcgggaaacagcaccaggaagctggtgacatatcgtctttcattgcgagaaacatcttacttatgtacatttctaagctatagcgtctacccttgtcagacccaggacgatgggtgtcacatctcctttctagtcaacctaagagaggaggaaatgccgcgatatatgttccaccctgtcatcacgaaggccaccacaatctatcccagaacagccggcacttcactcacgatgccccgatgctggattcctattgtcgcccttattagggcaagcggtgccagtagcagaatatgtcacctcaacaactcgatccacccctgcccattacatgggtaacatatccatggaggttcgatgtatactcgaggatacagtcgtccatcacgcccgcctacatacccattacatcagcatag

SEQ ID NO: 14 - DNA, 484 bp, Propionibacterium acnes
gttgcacaccagggggtcaacttggcgttttcagttcaaaattgattcaaactaacagttccatgccgggaaacagcaccaggaagctcgtgacatatcgtctttcattgcgagaaacatcttacttatgtacatttctaagctatagcgtctacccttgtcagacccaggacgatgggtgtcacatctcctttctagtcaacctaagagaggaggaaatgccgcgatatatgttccaccctgtcatcacgaaggccaccacaatctatcccagaacagccggcacttcactcacgatgccccgatgctggattcctattgtcgcccttattagggcaagcggtgccagtagcagaatatgtcacctcaacaactcgatccacccctgcccattacatgggtaacatatccatggaggttcgatgtatactcgaggatacagtcgtccatcacgcccgcctacatacccattacatcagcatag

SEQ ID NO: 15 - DNA, 484 bp, Propionibacterium acnes
gttgcacaccagggggtcaacttggcgtcctcagttcaaaattgattcaaactaacagttccatgccgggaaacagtaccaggaagctcgtgacatatcgtctttcattgcgagaaacatcttacttatgtacatttctaagctatagcgtctacccttgtcagacccaggacgatgggtgtcacatctcctttctagtcaacctaagagaggaggaaatgccgcgatatatgttccaccctgtcatcacgaaggccaccacaatctatcccagaacagccggcacttcactcacgatgccccgatgctggattcctattgtcgcccttattagggcaagcggtgccagtagcagaatatgtcacctcaacaactcgatccacccctgcccattacatgggtaacatatccatggaggttcgatgtatactcgaggatacagtcgtccatcacgcccgcctacatacccattacatcagcatag

SEQ ID NO: 16 - DNA, 484 bp, Propionibacterium acnes
gttgcacaccagggggtcaacttggcgtcctcagttcaaaattgattcaaactaacagttccatgccgggaaacagcaccaggaagctcgtgacatatcgtctttcattgcgagaaacatcttacttatgtacatttctaagctatagcgtctacccttgtcagacccaggacgatgggtgtcacatctcctttctagtcaacctaagagaggaggaaatgccgcgatatatgttccaccctgtcatcacgaaggccaccacaatctatcccagaacagccggcacttcactcacgatgccccgatgctggatccctattgtcgcccttattagggcaagcggtgccagtagcagaatatgtcacctcaacaactcgatccacccctgcccattacatgggtaacatatccatggaggttcgatgtatactcgaggatacagtcgtccatcacgcccgcctacatacccattacatcagcatag

SEQ ID NO: 17 - DNA, 484 bp, Propionibacterium acnes
gttgcacaccagggggtcaacttggcgtcctcagttcaaaattgattcaaactaacagttccatgtcgggaaacagcaccaggaagctcgtgacatatcgtctttcattgcgagaaacatcttacttatgtacatttctaagctatagcgtctacccttgtcagacccaggacgatgggtgtcacatctcctttctagtcaacctaagagaggaggaaatgccgcgatatatgttccaccctgtcatcacgaaggccaccacaatctatcccagaacagccggcacttcactcacgatgccccgatgctggattcctattgtcgcccttattagggcaagcggtgccggtagcagaatatgtcacctcaacaactcgatccacccctgcccattacatgggtaacatatccatggaggttcgatgtatactcgaggatacagtcgtccatcacgcccgcctacatacccattacatcagcatag

SEQ ID NO: 18 - DNA, 484 bp, Propionibacterium acnes
gttgcacaccagggggtcaacttggcgtcctcagttcaaaattgattcaaactaacagttccatgtcgggaaacagcaccaggaagctcgtgacatatcgtctttcattgcgagaaacatcttacttatgtacatttctaagctatagcgtctacccttgtcagacccaggacgatgggtgtcacatctcctttctagtcaacctaagagaggaggaaatgccgcgatatatgttccaccctgtcatcacgaaggccaccacaatctatcccagaacagccggcacttcactcacgatgccccgatgctggattcctattgtcgcccttattagggcaagcggtgccagtagcagaatatgccacctcaacaactcgatccacccctgcccattacatgggtaacatatccatggaggttcgatgtatactcgaggatacagtcgtccatcacgcccgcctacatacccattacatcagcatag

SEQ ID NO: 19 - DNA, 484 bp, Propionibacterium acnes
gttgcacaccagggggtcaacttggcgtcctcagttcaaaattgattcaaactaacagttccatgtcgggaaacagcaccaggaagctcgtgacatatcgtctttcattgcgagaaacatcttacttatgtacatttctaagctatagcgtctacccttgtcagacccaggacgatgggtgtcacatctcctttctagtcaacctaagagaggaggaaatgccgcgatatatgttccaccctgtcatcacgaaggccaccacaatctatcccagaacagccggcacttcactcacgatgccccgatgctggattcctattgtcgcccttattagggcaagcggtgccagtagcagaatatgtcacctcaacaactcgatcgacccctgcccattacatgggtaacatatccatggaggttcgatgtatactcgaggatacagtcgtccatcacgcccgcctacatacccattacatcagcatag

SEQ ID NO: 20 - DNA, 484 bp, Propionibacterium acnes
gttgcacaccagggggtcaacttggcgtcctcagttcaaaattgattcaaactaacagttccatgtcgggaaacagcaccaggaagctcgtgacatatcgtctttcattgcgagaaacatcttacttatgtacatttctaagctatagcgtctacccttgtcagacccaggacgatgggtgtcacatctcctttctagtcaacctaagagaggaggaaatgccgcgatatatgttccaccctgtcatcacgaaggccaccacaatctatcccagaacagccggcacttcactcacgatgccccgatgctggattcctattttcgcccttattagggcaagcggtgccagtagcagaatatgtcacctcaacaactcgatccacccctgcccattacatgggtaacatatccatggaggttcgatgtatactcgaggatacagtcgtccatcacgcccgcctacatacccattacatcagcatag

SEQ ID NO: 21 - DNA, 484 bp, Propionibacterium acnes
gttgcacaccagggggtcaacttggcgtcctcagttcaaaattgattcaaactaacagttccatgccgggaaacagcaccaggaagctcgtgacatatcgtctttcattgcgagaaacatcttacttatgtacatttctaagctatagcgtctacccttgtcagacccaggacgatgggtgtcacatctcctttctagtcaacctaagagaggaggaaatgccgcgatatatgttccaccctgtcatcacgaaggccaccacaatctatcccagaacagccggcacttcactcacaatgccccgatgctggattcctattgtcgcccttattagggcaagcggtgccagtagcagaatatgtcacctcaacaactcgatccacccctgcccattacatgggtaacatatccatggaggttcgatgtatactcgaggatacagtcgtccatcacgcccgcctacatacccattacatcagcatag

SEQ ID NO: 22 - DNA, 484 bp, Propionibacterium acnes
gttgcacaccagggggtcaacttggcgtcctcagttcaaaattgattcaaactaacagttccatgccgggaaacagcaccaggaagctcgtgacatatcgtctttcattgcgagaaacatcttacttatgtacatttctaagctatagcgtctacccttgtcagacccaggacgatgggtgtcacatctcctttctggtcaacctaagagaggaggaaatgccgcgatatatgttccaccctgtcatcacgaaggccaccacaatctatcccagaacagccggcacttcactcacgatgccccgatgctggattcctattgtcgcccttattagggcaagcggtgccagtagcagaatatgtcacctcaacaactcgatccacccctgcccattacatgggtaacatatccatggaggttcgatgtatactcgaggatacagtcgtccatcacgcccgcctacatacccattacatcagcatag

SEQ ID NO: 23 - DNA, 484 bp, Propionibacterium acnes
gttgcacaccagggggtcaacttggcgtcctcagttcaaaattgattcaaactaacagttccatgtcgggaaacagcaccaggaagctcgtgacatatcgtctttcattgcgagaaacatcttacttatgtacatttctaagctatagcgtctacccttgtcagacccaggacgatgggtgtcacatctcctttctagtcaacccaagagaggaggaaatgccgcgatatatgttccaccctgtcatcacgaaggccaccacaatctatcccagaacagccggcacttcactcacgatgccccgattctggattcctattgtcgcccttattagggcaagcggtgccagtagcagaatatgtcacctcaacaactcgatccacccctgcccattacatgggtaacatatccatggaggttcgatgtatactcgaggatacagtcgtccatcacgcccgcctacatacccattacatcagcatag

SEQ ID NO: 24 - DNA, 484 bp, Propionibacterium acnes
gttgcacaccagggggtcaacttggcgtcctcagttcaaaattgattcaaactaacagttccatgtcgggaaacagcaccaggaagctcgtgacatatcgtctttcattgcgagaaacatcttacttatgtacatttctaagctatagcgtctacccttgtcagacccaggacgatgggtgtcacatcccctttctagtcaacctaagagaggaggaaatgccgcgatatatgttccaccctgtcatcacgaaggccaccacaatctatcccagaacagccggcacttcactcacgatgccccgatgctggattcctattgtcgcccttattagggcaagcggtgccagtagcagaatatgtcacctcagcaactcgatccacccctgcccattacatgggtaacatatccatggaggttcgatgtatactcgaggatacagtcgtccatcacgcccgcctacatacccattacatcagcatag

SEQ ID NO: 25 - DNA, 484 bp, Propionibacterium acnes
gttgcacaccagggggtcaacttggcgtcctcagttcaaaattgattcaaactaacagttccatgtcgggaaacagcaccaggaagctcgtgacatatcgtctttcattgcgagaaacatcttacttatgtacatttctaagctatagcgtctacccttgtcagacccaggacgatgggtgtcacatcccctttctagtcaacctaagagaggaggaaatgccgcgatatatgttccaccctgtcatcacgaaggccaccacaatctatcccagaacagccggcacttcactcacgatgccccgatgctggattcctattgtcgcccttattagggcaagcggtgccagtagcagaatatgtcacctcaacaactcgatccacccctgcccattacatgggtaacatatccatggaggttcgatgtatactcgaggatacagtcgtccatcacgcccgcctacatacccattacatcagcatag

SEQ ID NO: 26 - DNA, 484 bp, Propionibacterium acnes
gttgcacaccagggggtcaacttggcgtcctcagttcaaaattgattcaaactaacagttccatgtcgggaaacagcaccaggaagctcgtgacatatcgtctttcattgcgagaaacatcttacttatgtacatttctaagctatagcgtctacccttgtcagacccatgacgatgggtgtcacatcccctttctagtcaacctaagagaggaggaaatgccgcgatatatgttccaccctgtcatcacgaaggccaccacaatctatcccagaacagccggcacttcactcacgatgccccgatgctggattcctattgtcgcccttattagggcaagcggtgccagtagcagaatatgtcacctcaacaactcgatccacccctgcccattacatgggtaacatatccatggaggttcgatgtatactcgaggatacagtcgtccatcacgcccgcctacatacccattacatcagcatag

SEQ ID NO: 27 - DNA, 484 bp, Propionibacterium acnes
gttgcacaccagggggtcaacttggcgtccttagttcaaaattgattcaaactaacagttccatgtcgggaaacagcaccaggaagctcgtgacatatcgtctttcattgcgagaaacatcttacttatgtacatttctaagctatagcgtctacccttgtcagacccaggacgatgggtgtcacatcccctttctagtcaacctaagagaggaggaaatgccgcgatatatgttccaccctgtcatcacgaaggccaccacaatctatcccagaacagccggcacttcactcacgatgccccgatgctggattcctattgtcgcccttattagggcaagcggtgccagtagcagaatatgtcacctcaacaactcgatccacccctgcccattacatgggtaacatatccatggaggttcgatgtatactcgaggatacagtcgtccatcacgcccgcctacatacccattacatcagcatag

SEQ ID NO: 28 - DNA, 484 bp, Propionibacterium acnes
gttgcacaccagggggtcaacttggcgtcctcagttcaaaattgattcaaactaacagttccatgtcgggaaacagcaccaggaagctcgtgacatatcgtctttcattgcgagaaacatcttacttatgtacatttctaagctatagcgtctacccttgtcagacccaggacgatgggtgtcacatcccctttctagtcaacctaagagaggaggaaatgccgcgatatatgttccaccctgtcatcacgaaggccaccacaatctatcccagaacagccggcacttcactcacgatgccccgatgctggattcctattgtcgcccttattagggcaagcggtgccagtagcagaatatgtcacctcaacaactcgatccacccctgcccattacatgggtaacatatccatggaggttcgatgtatactcgaggatacagtcgtccatcacgcccgcctacatacccattacatctgcatag

SEQ ID NO: 29 - DNA, 484 bp, Propionibacterium acnes
gttgcacaccagggggtcaacttggcgtcctcagttcaaaattgattcaaactaacagttccatgtcgggaaacagcaccaggaaactcgtgacatatcgtctttcattgcgagaaacatcttacttatgtacatttctaagctatagcgtctacccttgtcagacccaggacgatgggtgtcacatcccctttctagtcaacctaagagaggaggaaatgccgcgatatatgttccgccctgtcatcacgaagaccaccacaatctatcccagaacagccggcacttcactcacgatgccccgatgctggattcctattgtcgcccttattagggcaagcggtgccagtagcagaatatgtcacctcaacaactcgatccacccctgcccattacatgggtaacatatccatggaggttcgatgtatacttgaggatacagtcgtccatcacgcccacctacatacccattacatcagcatag

SEQ ID NO: 30 - DNA, 484 bp, Propionibacterium acnes
gttgcacaccagggggtcaacttggcgtcctcagttcaaaattgattcaaactaacagttccatgtcgggaaacagcaccaggaaactcgtgacatatcgtctttcattgcgagaaacatcttacttatgtacatttctaagctatagcgtctacccttgtcagacccaggacgatgggtgtcacatcccctttctagtcaacctaagagaggaggaaacgccgcgatatatgttccgccctgtcatcacgaagaccaccacaatctatcccagaacagccggcacttcactcacgatgccccgatgctggattcctattgtcgcccttattagggcaagcggtgccagtagcagaatatgtcacctcaacaactcgatccacccctgcccattacatgggtaacatatccatggaggttcgatgtatacttgaggatacagtcgtccatcacgcccacctacatacccattacatcagcatag

SEQ ID NO: 31 - DNA, 484 bp, Propionibacterium acnes
gttgcacaccagggggtcaacttggcgtcctcagttcaaaattgattcaaactaacagttccatgtcgggaaacagcaccaggaaactcgtgacatatcgtctttcattgcgagaaacatcttacttatgtacatttctaagctatagcgtctacctttgtcagacccaggacgatgggtgtcacatcccctttctagtcaacctaagagaggaggaaatgccgcgatatatgttccgccctgtcatcacgaagaccaccacaatctatcccagaacagccggcacttcactcacgatgccccgatgctggattcctattgtcgcccttattagggcaagcggtgccagtagcagaatatgtcacctcaacaactcgatccacccctgcccattacatgggtaacatatccatggaggttcgatgtatacttgaggatacagtcgtccatcacgcccacctacatacccattacatcagcatag

SEQ ID NO: 32 - DNA, 484 bp, Propionibacterium acnes
gttgcacaccagggggtcaacttggcgtcctcagttcaaaattgatttaaactaacagttccatgtcgggaaacagcaccaggaagctcgtgacatatcgtctttcattgcgagaaacatcttacttatgtacatttctaagctatagcgtctacccttgtcagacccaggacgatggatgtcacatcccctttctagtcaacctaagagaggaggaaatgccgcgatatatgttccaccctgtcatcacgaaggccaccacaatctatcccagaacagccggcacctcactcacgatgccccgatgctggattcctattgtcgcccttattagggcaagcggtgccagtagcagaatatgtcacctcaacaactcgatccacccctgcccattacatgggtaacatatccatggaggttcgatgtatattcgagaatacagtcgtccatcacgcccgcctacatacccattacatcagcatag

SEQ ID NO: 33 - DNA, 484 bp, Propionibacterium acnes
gttgcacaccagggggtcaacttggcgtcctcagttcaaaattgatttaaactaacagttccatgtcgggaaacagcaccagaaagctcgtgacatatcgtctttcattgcgagaaacatcttacttatgtacatttctaagctatagcgtctacccttgtcagacccaggacgatggatgtcacatcccctttctagtcaacctaagagaggaggaaatgccgcgatatatgttccaccctgtcatcacgaaggccaccacaatctatcccagaacagccggcacctcactcacgatgccccgatgctggattcctattgtcgcccttattagggcaagcggtgccagtagcagaatatgtcacctcaacaactcgatccacccctgcccattacatgggtaacatatccatggaggttcgatgtatattcgaggatacagtcgtccatcacgcccgcctacatacccattacatcagcatag

SEQ ID NO: 34 - DNA, 484 bp, Propionibacterium acnes
gttgcacaccagggggtcaacttggcgtcctcagttcaaaattgatttaaactaacagttccatgtcgggaaacagcaccaggaagctcgtgacatatcgtctttcattgcgagaaacatcttacttatgtacatttctaagctatagcgtctacccttgtcagacccaggacgatggatgtcacatcccctttctagtcaacctaagagaggaggaaatgccgcgatatatgttccaccctgtcatcacgaaggccaccacaatctatcccagaacagccggcacctcactcacgatgccccgatgctggattcctattgtcgcccttattagggcaagcggtgccagtagcagaatatgtcacctcaacaactcgatccacccctgcccattacatgggtaacatatccatggaggttcgatgtatattcgaggatacagtcgtccatcacgcccgcctacatacccattacatcagcatag

SEQ ID NO: 35 - DNA, 484 bp, Propionibacterium acnes
gttgcacaccagggggtcaacttggcgtcctcagttcaaaattgatttaaactaacagttccatgtcgggaaacagcaccaggaagctcgtgacatatcgtctttcattgcgagaaacatcttacttatgtacatttctaagctatagcgtctacccttgtcagacccaggacgatggatgtcacatcccctttctagtcaacctaagagaggaggaaatgccgcgatatatgttccaccctgtcatcacgaaggccaccacaatctatcccagaacagccggcacctcactcacgatgccccgatgctggattcctattgtcgcccttattagggcaagcggtgccagtagcagaatatgtcacctcaacaactcgatccacccctgcccattacatgggtaacatatccatgaaggttcgatgtatattcgaggatacagtcgtccatcacgcccgcctacatacccattacatcagcatag

SEQ ID NO: 36 - DNA, 484 bp, Propionibacterium acnes
gttgcacaccagggggtcaacttggcgtcctcagttcaaaattgatttaaactaacagtttcatgtcgggaaacagcaccaggaagctcgtgacatatcgtctttcattgcgagaaacatcttacttatgtacatttctaagctatagcgtctacccttgtcagacccaggacgatggatgtcacatcccctttctagtcaacctaagagaggaggaaatgccgcgatatatgttccaccctgtcatcacgaaggccaccacaatctatcccagaacagccggcacctcactcacgatgccccgatgctggattcctattgtcgcccttattagggcaagcggtgccagtagcagaatatgtcacctcaacaactcgatccacccctgcccattacatgggtaacatatccatggaggttcgatgtatattcgaggatacagtcgtccatcacgcccgcctacatacccattacatcagcatag

SEQ ID NO: 37 - DNA, 484 bp, Propionibacterium acnes
gttgcacaccagggggtcaacttggcgtcctcagttcaaaattgatttaaactaacagttccatgtcgggaaacagcaccaggaagctcgtgacatatcgtctttcattgcgagaaacatcttacttatgtacatttctaagctatagcgtctacccttgtcagacccaggacgatggatgtcacatcccctttctagtcaacctaagagaggaggaaattccgcgatatatgttccaccctgtcatcacgaaggccaccacaatctatcccagaacagccggcacctcactcacgatgccccgatgctggattcctattgtcgcccttattagggcaagcggtgccagtagcagaatatgtcacctcaacaactcgatccacccctgcccattacatgggtaacatatccatggaggttcgatgtatattcgaggatacagtcgtccatcacgcccgcctacatacccattacatcagcatag

SEQ ID NO: 38 - DNA, 484 bp, Propionibacterium acnes
gttgcacaccagagggtcaacttggcgtcctcagttcaaaattgatttaaactaacagttccatgtcgggaaacagcaccaggaagctcgtgacatatcgtctttcattgcgagaaacatcttacttatgtacatttctaagctatagcgtctacccttgtcagacccaggacgatggatgtcacatcccctttctagtcaacctaagagaggaggaaatgccgcgatatatgttccaccctgtcatcacgaaggccaccacaatctatcccagaacagccggcacctcactcacgatgccccgatgctggattcctattgtcgcccttattagggcaagcggtgccagtagcagaatatgtcacctcaacaactcgatccacccctgcccattacatgggtaacatatccatggaggttcgatgtatattcgaggatacagtcgtccatcacgcccgcctacatacccattacatcagcatag

SEQ ID NO: 39 - DNA, 484 bp, Propionibacterium acnes
gttgcacaccagggggtcaacttggcgtcctcagttcaaaattgatttaaactaacagttccatgtcgggaaacagcaccaggaagctcgtgacatatcgtctttcattgcgagaaacatcttacttatgtacatttctaagctatagcgtctacccttgtcagacccaggacgatggatgtcacatcccctttctagtcaacctaagagaggaggaaatgccgcgatatatgttccaccctgtcatcacgaaggccaccacaatctatcccagaacagccggcgcctcactcacgatgccccgatgctggattcctattgtcgcccttattagggcaagcggtgccagtagcagaatatgtcacctcaacaactcgatccacccctgcccattacatgggtaacatatccatggaggttcgatgtatattcgaggatacagtcgtccatcacgcccgcctacatacccattacatcagcatag

SEQ ID NO: 40 - DNA, 484 bp, Propionibacterium acnes
gttgcacaccagggggtcaacttggcgtcctcagttcaaaatagatttaaactaacagttccatgtcgggaaacagcaccaggaagctcgtgacatatcgtctttcattgcgagaaacatcttacttatgtacatttctaagctatagcgtctacccttgtcagacccaggacgatggatgtcacatcccctttctagtcaacctaagagaggaggaaatgccgcgatatatgttccaccctgtcatcacgaaggccaccacaatctatcccagaacagccggcacctcactcacgatgccccgatgctggattcctattgtcgcccttattagggcaagcggtgccagtagcagaatatgtcacctcaacaactcgatccacccctgcccattacatgggtaacatatccatggaggttcgatgtatattcgaggatacagtcgtccatcacgcccgcctacatacccattacatcagcatag

SEQ ID NO: 41 - DNA, 484 bp, Propionibacterium acnes
gttgcacaccagggggtcaacttggcgtcctcagttcaaaattgattcaaactaacagttccatgtcgggaaacagcaccaggaagctcgtgacatatcgtctttcattgcgagaaacatcttacttatgtatatttctaagctatagcgtctacccttgtcagacccaggacgatgggtgtcacatcccctttctagtcaacctaagagaggaggaaatgccgcgatatatgttccaccctgtcatcacgaacgccaccacaatctatcccagaacagccggcacttcactcacgatgccccgattctggattcctattgtcgcccttattagggcaagcggtgccagtagcagaatatgtcacctcaacaactcgatccacccctgcccattacatgggtaacatatccatggaggttcgatgtatactcgaggatacagtcgtccatcacgcccgcctacatacccattacatcagcatag

SEQ ID NO: 42 - DNA, 484 bp, Propionibacterium acnes
gttgcacaccagggggtcaacttggcgtcctcagttcaaaattgattcaaactaacagttccatgtcgggaaacagcaccaggaagctcgtgacatatcgtctttcattgcgagaaacatcttacttatgtatatttctaagctatagcgtctacccttgtcagacccaggacgatgggtgtcacatcccctttctagtcaacctaagagaggaggaaatgccgcgatatatgttccaccctgtcatcacgaacgccaccacaatctatcccagaacagccggcacttcactcacgatgccccgattctggattcctattgtcgcccttattagggcaagcggtgccagtagcagaatatgtcacctcaacaactcgatccacccctgcccattacatgggtaacatatccatggaggttcgatgtatactcgaggatacagtcgtccatcacgcccgcctacatacccattacaccagcatag

SEQ ID NO: 43 - DNA, 484 bp, Propionibacterium acnes
gttgcacaccagggggtcaacttggcgtcctcagttcaaaattgattcaaactaacagttccatgtcgggaaacagcaccaggaagctcgtgacatatcgtctttcattgcgagaaacatcttacttatgtatatttctaagctatagcgtctacccttgtcagacccaggacgatgggtgtcacatcccctttctagtcaacctaagagaggaggaaatgccgcgatatatgttccaccctgtcatcacgaacgccaccacaatctatcccagaacagccggcacttcactcacgatgccccgattctggattcctattgtcgcccttattagggcaagcggtgccagtagcagaatatgtcacctaaacaactcgatccacccctgcccattacatgggtaacatatccatggaggttcgatgtatactcgaggatacagtcgtccatcacgcccgcctacatacccattacatcagcatag

SEQ ID NO: 44 - DNA, 484 bp, Propionibacterium acnes
gttgcacaccagggggtcaacttggcgtcctcagttcaaaattgattcaaactaacagttccatgtcgggaaacagcaccaggaagctcgtgacatatcgtctttcattgcgagaaacatcttacttatgtacatttctaagctatagcgtctacccttgtcagacccaggacgatgggtgtcacatcccctttctagtcaacctaagagaggaggaaatgccgcgatatatgttccaccctgtcatcacgaacgccaccacaatctatcccagaacagccggcacttcactcacgatgccccgatgctggattcctattgtcgcccttattagggcaagcggtgccagtagcagaatatgtcacctcaacaactcgatccacccctgcccattacatgggtaacatatccatggaggttcgatgtatactcgaggatacagtcgtccatcacgcccgcctacatacccattacatcagcatag

SEQ ID NO: 45 - DNA, 484 bp, Propionibacterium acnes
gttgcacaccagggggtcaacttggcgtcctcagttcaaaattgattcaaactaacagttccatgtcgggaaacagcaccaggaagctcgtgacatatcgtctttcattgcgagaaacatcttacttatgtacatttctaagctatagcgtctacccttgtcagacccaggacgatgggtgtcacatcccctttctagtcaacctaagagaggaggaaatgccgcgatatatgttccaccctgtcatcacgaacgccaccacaatctatcccagaacagccggcacttcactcacgatgccccgatgctagattcctattgtcgcccttattagggcaagcggtgccagtagcagaatatgtcacctcaacaactcgatccacccctgcccattacatgggtaacatatccatggaggttcgatgtatactcgaggatacagtcgtccatcacgcccgcctacatacccattacatcagcatag

SEQ ID NO: 46 - DNA, 484 bp, Propionibacterium acnes
gttacacaccagggggtcaacttggcgtcctcagttcaaaattgattcaaactaacagttccatgtcgggaaacagcaccaggaagctcgtgacatatcgtctttcattgcgagaaacatcttacttatgtacatttctaagctatagcgtctacccttgtcagacccaggacgatgggtgtcacatcccctttctagtcaacctaagagaggaggaaatgccgcgatatatgttccaccctgtcatcacgaacgccaccacaatctatcccagaacagccggcacttcactcacgatgccccgatgctggattcctattgtcgcccttattagggcaagcggtgccagtagcagaatatgtcacctcaacaactcgatccacccctgcccattacatgggtaacatatccatggaggttcgatgtatactcgaggatacagtcgtccatcacgcccgcctacatacccattacatcagcatag

SEQ ID NO: 47 - DNA, 484 bp, Propionibacterium acnes
gttgcacaccagggggtcaacttggcgtcctcagttcaaaattgattcaaactaacagttccatgtcgggaaacagcaccaggaagctcgtgacatatcgtctttcattgcgagaaacatcttacttatgtatatttctaagctatagcgtctacccttgtcagacccaggacgatgggtgtcacatcccctttctagtcaacctaagagaggaggaaatgccgcgatatatgttccaccctgtcatcacgaacgccaccacaatctatcccagaacagccggcacttcactcacgatgccccgattctggattcctattgtcgcccttattagggcaagcggtgccagtagcagaatatgtcacctcaacaactcgatccacccctgcccattacatgggtaacatatccatggaggttcgatgtatactcgaggatacagtcgtccatcaagcccgcctacatacccattacatcagcatag

SEQ ID NO: 48 - DNA, 484 bp, Propionibacterium acnes
gttgcacaccagggggtcaacttggcgtcctcagttcaaaattgattcaaactaacagttccatgtcggaaaacagcaccaggaagctcgtgacatatcgtctttcattgcgagaaacatcttacttatgtacatttctaagctatagcgtctacccttgtcagacccaggacgatgggtgtcacatcccctttctagtcaacctaagagaggaggaaatgccgcgatatatgttccaccctgtcatcacgaacgccaccacaatctatcccagaacagccggcacttcactcacgatgccccgatgctggattcctattgtcgcccttattagggcaagcggtgccagtagcagaatatgtcacctcaacaactcgatccacccctgcccattacatgggtaacatatccatggaggttcgatgtatactcgaggatacagtcgtccatcacgcccgcctacatacccattacatcagcatag

SEQ ID NO: 49 - DNA, 484 bp, Propionibacterium acnes
gttgcacaccagggggtcaacttggcgtcctcagttcaaaattgattcaaactaacagttccatgtcgggaaacagcaccaggaagctcgtgacatatcgtctttcattgcgagaaacatcttacttatgtacatttctaagctatagcgtctacccttgtcagacccaggacgatgggtgtcacatcccctttctagtcaacctaagagaggaggaaatgccgcgatatatgttccaccctgtcatcacgaacgccaccacaatctatcccagaacagccggcacttcactcacgatgccccgatgctggattcctattgtcgcccttattagggcaagcgatgccagtagcagaatatgtcacctcaacaactcgatccacccctgcccattacatgggtaacatatccatggaggttcgatgtatactcgaggatacagtcgtccatcacgcccgcctacatacccattacatcagcatag

SEQ ID NO: 50 - DNA, 484 bp, Propionibacterium acnes
gttgcacaccagggggtcaacttggcgtcctcagttcaaaattgattcaaactaacagttccatgtcgggaaacagcaccaggaagctcgtgacatatcgtctttcattgcgagaaacatcttacttatgtacatttctaagctatagcgtctacccttgtcagacccaggacgatgggtgtcacaccccctttctagtcaacctaagagaggaggaaatgccgcgatatatgttccaccctgtcatcacgaacgccaccacaatctatcccagaacagccggcacttcactcacgatgccccgatgctggattcctattgtcgcccttattagggcaagcggtgccagtagcagaatatgtcacctcaacaactcgatccacccctgcccattacatgggtaacatatccatggaggttcgatgtatactcgaggatacagtcgtccatcacgcccgcctacatacccattacatcagcatag

SEQ ID NO: 51 - DNA, 484 bp, Propionibacterium acnes
gttgcacaccagggggtcaacttggcgtcctcagttcaaaattgattcaaactaacagttccatgtcgggaaacagcaccaggaagctcgtgacatatcgcctttcattgcgagaaacatcttacttatgtacatttctaagctatagcgtctacccttgtcagacccaggacgatgggtgtcacatcccctttctagtcaacctaagagaggaggaaatgccgcgatatatgttccaccctgtcatcacgaacgccaccacaatcgatcccagaacagccggcacttcactcacgatgccccgatgctggattcctattgtcgcccttattagggcaagcggtgccagtagcagaatatgtcacctcaacaactcgatccacccctgcccattacatgggtaacatatccatggaggttcgatgtatactcgaggatacagtcgtccatcacgcccgcctacatacccattacatcagcatag

SEQ ID NO: 52 - DNA, 484 bp, Propionibacterium acnes
gttgcacaccagggggtcaacttggcgtcctcagttcaaaattgattcaaactaacagttccatgtcgggaaacagcaccaggaagctcgtgacatatcgtctttcattgcgagaaacatcttacttatgtacatttctaagctatatcgtctacccttgtcagacccaggacgatggatgtcacatcccctttctagtcaacctaagagaggaggaaatgccgcgatatatgttccaccctgtcatcacgaaggccaccacaatctatcccagaacagccggcacttcactcacgatgccccgatgctggattcctattgtcgcccttattagggcaagcggtgccagtagcagaatatgtcacctcaacaactcgatccacccctgcccattacatgggtaacatatccatggaggttcgatgtatattcgaggatacagtcgtccatcacgcccgcctacatacccattacatcagcatag

SEQ ID NO: 53 - DNA, 484 bp, Propionibacterium acnes
gttgcacaccagggggtcaacttggcgtcctcagttcaaaattgattcaaactaacagttccatgtcgggaaacagcaccaggaagctcgtgacatatcgtctttcattgcgagaaacatcttacttatgtacatttctaagctatatcgtctacccttgtcagacccaggacgatggatgtcacatcccctttctagtcaacctaagagaggaggaaatgccgcgatatatgttccaccctgtcatcacgaaggccaccacaatctatcccagaacagccggcacttcactcacgatgccccgatgctggattcctattgtcgccctcattagggcaagcggtgccagtagcagaatatgtcacctcaacaactcgatccacccctgcccattacatgggtaacatatccatggaggttcgatgtatattcgaggatacagtcgtccatcacgcccgcctacatacccattacatcagcatag

SEQ ID NO: 54 - DNA, 484 bp, Propionibacterium acnes
gttgcacaccagggggtcaacttggcgtcctcagttcaaaattgattcaaactaacagttccatgtcgggaaacagcaccaggaagctcgtgacatatcgtctttcattgcgagaaacatcttacttatgtacatttctaagctatatcgtccacccttgtcagacccaggacgatggatgtcacatcccctttctagtcaacctaagagaggaggaaatgccgcgatatatgttccaccctgtcatcacgaaggccaccacaatctatcccagaacagccggcacttcactcacgatgccccgatgctggattcctattgtcgcccttattagggcaagcggtgccagtagcagaatatgtcacctcaacaactcgatccacccctgcccattacatgggtaacatatccatggaggttcgatgtatattcgaggatacagtcgtccatcacgcccgcctacatacccattacatcagcatag

SEQ ID NO: 55 - DNA, 484 bp, Propionibacterium acnes
gttgcacaccagggggtcaacttggcgtcctcagttcaaaattgattcaaactaacagttccatgtcgggaaacagcaccaggaagctcgtgacatatcgtctttcattgcgagaaacatcttacttatgtacatttctaagctatatcgtctacccttgtcagacccgggacgatggatgtcacatcccctttctagtcaacctaagagaggaggaaatgccgcgatatatgttccaccctgtcatcacgaaggccaccacaatctatcccagaacagccggcacttcactcacgatgccccgatgctggattcctattgtcgcccttattagggcaagcggtgccagtagcagaatatgtcacctcaacaactcgatccacccctgcccattacatgggtaacatatccatggaggttcgatgtatattcgaggatacagtcgtccatcacgcccgcctacatacccattacatcagcatag

SEQ ID NO: 56 - DNA, 484 bp, Propionibacterium acnes
gttgcacaccagggggtcaacttggcgtcctcagttcaaaattgattcaaactaacagttccatgtcgggaaacagcaccaggaagctcgtgacatatcgtctttcattgcgagaaacatcttacttatgtacatttctaagccatatcgtctacccttgtcagacccaggacgatggatgtcacatcccctttctagtcaacctaagagaggaggaaatgccgcgatatatgttccaccctgtcatcacgaaggccaccacaatctatcccagaacagccggcacttcactcacgatgccccgatgctggattcctattgtcgcccttattagggcaagcggtgccagtagcagaatatgtcacctcaacaactcgatccacccctgcccattacatgggtaacatatccatggaggttcgatgtatattcgaggatacagtcgtccatcacgcccgcctacatacccattacatcagcatag

SEQ ID NO: 57 - DNA, 484 bp, Propionibacterium acnes
gttgcacaccagggggtcaacttggtgtcctcagttcaaaattgattcaaactaacggttccgtgtcgggaaacagcaccagaaaactcgtgacatatcgtctttcattgcgagaaacatcttacttatacacatttctaagctatattgtctacccctgtcagacccaggacgatgggtgtcatatcccctttccagtcaacctaagaagggaggaaatgccgcgatatatgttccgccctgtcatcatgaatgccaccacaatctatcccggaacagccgtacttcacccaccatgccccgatgctggattcctattgtcgcccttattagagcaagcggtgccagcagcagaatatttcacctcagcaactcgatccgctcctgcccattacatgggtaacatatccatggaggtacgatgtatgcatcgaggatgcagtcgtctactatgcccgcctacatacccattccatcagcatag

SEQ ID NO: 58 - DNA, 484 bp, Propionibacterium acnes
gttgcacaccagggggtcaacttggtgtcctcagttcaaaattggttcaaactaacggttccgtgtcgggaaacagcaccagaaaactcgtgacatatcgtctttcattgcgagaaacatcttacttatacacatttctaagctatattgtctacccctgtcagacccaggacgatgggtgtcatatcccctttccagtcaacctaagaagggaggaaatgccgcgatatatgttccgccctgtcatcatgaatgccaccacaatctatcccggaacagccgtacttcacccaccatgccccgatgctggattcctattgtcgcccttattagagcaagcggtgccagcagcagaatatttcacctcagcaactcgatccgctcctgcccattacatgggtaacatatccatggaggtacgatgtatgcatcgaggatgcagtcgtctactatgcccgcctacatacccattccatcagcatag

SEQ ID NO: 59 - DNA, 483 bp, Propionibacterium acnes
gttgcacaccagggggtcaacttggtgtcctcagttcaaaattgattcaaactaacggttccgtgtcgggaaacagcaccagaaaactcgtgacatatcgtctttcattgcgagaaacatcttacttatacacatttctaagctatatgtctacccctgtcagacccaggacgatgggtgtcatatcccctttccagtcaacctaagaagggaggaaatgccgcgatatatgttccgccctgtcatcatgaatgccaccacaatctatcccggaacagccgtacttcacccaccatgccccgatgctggattcctattgtcgcccttattagagcaagcggtgccagcagcagaatatttcacctcagcaactcgatccgctcctgcccattacatgggtaacatatccatggaggtacgatgtatgcatcgaggatgcagtcgtctactatgcccgcctacatacccattccatcagcatag

SEQ ID NO: 60 - DNA, 484 bp, Propionibacterium acnes
gttgcacaccagggggtcaacttggtgtcctcagttcaaaattgattcaaactaacggttccgtgtcgggaaacagcaccagaaaactcgtaacatatcgtctttcattgcgagaaacatcttacttatacacatttctaagctatattgtctacccctgtcagacccaggacgatgggtgtcatatcccctttccagtcaacctaagaagggaggaaatgccgcgatatatgttccgccctgtcatcatgaatgccaccacaatctatcccggaacagccgtacttcacccaccatgccccgatgctggattcctattgtcgcccttattagagcaagcggtgccagcagcagaatatttcacctcagcaactcgatccgctcctgcccattacatgggtaacatatccatggaggtacgatgtatgcatcgaggatgcagtcgtctactatgcccgcctacatacccattccatcagcatag

SEQ ID NO: 61 - DNA, 484 bp, Propionibacterium acnes
gttgcacaccagggggtcaacttggtgtcctcagttcaaaattgattcaaactaacggttccgtgtcgggaaacagcaccagaaaactcgtgacatatcgtctttcattgcgagaaacatcttacttatacacatttctaagctatattgtctacccctgtcagacccaggacgatgggtgtcatatcccctttccagtcaacctaagaagggaggaaatgccgcgatatatgttccgccctgtcatcatgaatgccaccacaatctatcccggaacagccgtacttcacccaccatgcctcgatgctggattcctattgtcgcccttattagagcaagcggtgccagcagcagaatatttcacctcagcaactcgatccgctcctgcccattacatgggtaacatatccatggaggtacgatgtatgcatcgaggatgcagtcgtctactatgcccgcctacatacccattccatcagcatag

SEQ ID NO: 62 - DNA, 484 bp, Propionibacterium acnes
gttgcacaccagggggtcaacttggtgtcctcagttcaaaattgattcaaactaacggttccgtgtcgggaaacagcaccagaaaactcgtgacatatcgtctttcattgcgagaaacatcttatttatacacatttctaagctatattgtctacccctgtcagacccaggacgatgggtgtcatatcccctttccagtcaacctaagaagggaggaaatgccgcgatatatgttccgccctgtcatcatgaatgccaccacaatctatcccggaacagccgtacttcacccaccatgccccgatgctggattcctattgtcgcccttattagagcaagcggtgccagcagcagaatatttcacctcagcaactcgatccgctcctgcccattacatgggtaacatatccatggaggtacgatgtatgcatcgaggatgcagtcgtctactatgcccgcctacatacccattccatcagcatag

SEQ ID NO: 63 - DNA, 484 bp, Propionibacterium acnes
gttgcacaccagggggtcaacttggtgtcctcagttcaaaattgattcaaactaacggttccgtgtcgggaaacagcaccagaaaactcgtgacatatcgtctttcattgcgagaaacatcttacttatacacatttctaagctatattgtctacccctgtcagacccaggacgatgggtgtcatatcccctttccagtcaacctaagaaggaaggaaatgccgcgatatatgttccgccctgtcatcatgaatgccaccacaatctatcccggaacagccgtacttcacccaccatgccccgatgctggattcctattgtcgcccttattagagcaagcggtgccagcagcagaatatttcacctcagcaactcgatccgctcctgcccattacatggttaacatatccatggaggtacgatgtatgcatcgaggatgcagtcgtctactatgcccgcctacatacccattccatcagcatag

SEQ ID NO: 64 - DNA, 484 bp, Propionibacterium acnes
attgcacaccagggggtcaacttggtgtcctcagttcaaaattggttcaaactaacggttccgtgtcgggaaacagcaccagaaaactcgtgacatatcgtctttcattgcgagaaacatcttacttatacacatttctaagctatattgtctacccctgtcagacccaggacgatgggtgtcatatcccctttccagtcaacctaagaagggaggaaatgccgcgatatatgttccgccctgtcatcatgaatgccaccacaatctatcccggaacagccgtacttcacccaccatgccccgatgctggattcctattgtcgcccttattagagcaagcggtgccagcagcagaatatttcacctcagcaactcgatccgctcctgcccattacatgggtaacatatccatggaggtacgatgtatgcatcgaggatgcagtcgtctactatgcccgcctacatacccattccatcagcatag

SEQ ID NO: 65 - DNA, 484 bp, Propionibacterium acnes
gttgcacaccagggggtcaacttggtgtcctcagttcaaaattggttcaaactaacggttccgtgtcgggaaacagcaccagaaaactcgtgacatatcgtctttcattgcgagaaacatcttacttatacacatttctaagctatattgtctacccctgtcagacccaggacgatgggtgtcatatcccctttccagtcaacctaagaagggaggaaatgccgcgatatatgttccgccctgtcatcatgaatgccaccacaatctatcccggaacagccgtacttcacccaccatgccccgatgctggattcctatggtcgcccttattagagcaagcggtgccagcagcagaatatttcacctcagcaactcgatccgctcctgcccattacatgggtaacatatccatggaggtacgatgtatgcatcgaggatgcagtcgtctactatgcccgcctacatacccattccatcagcatag

SEQ ID NO: 66 - DNA, 483 bp, Propionibacterium acnes
gttgcacaccagggggtcaacttggtgtcctcagttcaaaattgattcaaactaacggttccgtgtcgggaaacagcaccagaaaactcgtgacatatcatctttcattgcgagaaacatcttacttatacacatttctaagctatatgtctacccctgtcagacccaggacgatgggtgtcatatcccctttccagtcaacctaagaagggaggaaatgccgcgatatatgttccgccctgtcatcatgaatgccaccacaatctatcccggaacagccgtacttcacccaccatgccccgatgctggattcctattgtcgcccttattagagcaagcggtgccagcagcagaatatttcacctcagcaactcgatccgctcctgcccattacatgggtaacatatccatggaggtacgatgtatgcatcgaggatgcagtcgtctactatgcccgcctacatacccattccatcagcatag

SEQ ID NO: 67 - DNA, 484 bp, Propionibacterium acnes
gttgcacaccagggggtcaacttggtgtcctcagttcaaaattggttcaaactaacggttccgtgtcgggaaacagcaccagaaaactcgtgacatgtcgtctttcattgcgagaaacatcttacttatacacatttctaagctatattgtctacccctgtcagacccaggacgatgggtgtcatatcccctttccagtcaacctaagaagggaggaaatgccgcgatatatgttccgccctgtcatcatgaatgccaccacaatctatcccggaacagccgtacttcacccaccatgccccgatgctggattcctattgtcgcccttattagagcaagcggtgccagcagcagaatatttcacctcagcaactcgatccgctcctgcccattacatgggtaacatatccatggaggtacgatgtatgcatcgaggatgcagtcgtctactatgcccgcctacatacccattccatcagcatag

SEQ ID NO: 68 - DNA, 484 bp, Propionibacterium acnes
gttgcacaccagggggtcaacttggtgtcctcagttcaaaattggttcaaactaacggttccgtgtcgggaaacagcaccagaaaactcgtgacatatcgtctttcattgcgagaaacatcttacttatacacatttctaagctatactgtctacccctgtcagacccaggacgatgggtgtcatatcccctttccagtcaacctaagaagggaggaaatgccgcgatatatgttccgccctgtcatcatgaatgccaccacaatctatcccggaacagccgtacttcacccaccatgccccgatgctggattcctattgtcgcccttattagagcaagcggtgccagcagcagaatatttcacctcagcaactcgatccgctcctgcccattacatgggtaacatatccatggaggtacgatgtatgcatcgaggatgcagtcgtctactatgcccgcctacatacccattccatcagcatag

SEQ ID NO: 69 - DNA, 484 bp, Propionibacterium acnes
gttgcacaccagggggtcaacttggtgtcctcagttcaaaattggttcaaactaacggttccgtgtcgggaaacagcaccagaaaacttgtgacatatcgtctttcattgcgagaaacatcttacttatacacatttctaagctatattgtctacccctgtcagacccaggacgatgggtgtcatatcccctttccagtcaacctaagaagggaggaaatgccgcgatatatgttccgccctgtcatcatgaatgccaccacaatctatcccggaacagccgtacttcacccaccatgccccgatgctggattcctattgtcgcccttattagagcaagcggtgccagcagcagaatatttcacctcagcaactcgatccgctcctgcccattacatgggtaacatatccatggaggtacgatgtatgcatcgaggatgcagtcgtctactatgcccgcctacatacccattccatcagcatag

SEQ ID NO: 70 - DNA, 484 bp, Propionibacterium acnes
gttgcacaccagggggtcaacttggtgtcctcagttcaaaattggttcaaactaacggttccgtgtcgggaaacagcaccagaaaactcatgacatatcgtctttcattgcgagaaacatcttacttatacacatttctaagctatattgtctacccctgtcagacccaggacgatgggtgtcatatcccctttccagtcaacctaagaagggaggaaatgccgcgatatatgttccgccctgtcatcatgaatgccaccacaatctatcccggaacagccgtacttcacccaccatgccccgatgctggattcctattgtcgcccttattagagcaagcggtgccagcagcagaatatttcacctcagcaactcgatccgctcctgcccattacatgggtaacatatccatggaggtacgatgtatgcatcgaggatgcagtcgtctactatgcccgcctacatacccattccatcagcatag

SEQ ID NO: 71 - DNA, 484 bp, Propionibacterium acnes
gttgcacaccagggggtcaacttggtgtcctcagttcaaaattgattcaaactaacggttccgtatcgggaaacagcaccagaaaactcgggacatatcgtctttcattgcgagaaaaatcttacttatgcgcatttctaagctatagcgtctacccttgtcagacccaggacgatgagtgtcacatcccctttccagtcaacctaagagaggaggaaatgccgcgatatatgctccgccctgtcatcacgaaagccaccacaatctatcccagaacagccggcacttcactcacgatgccccgatgctggattcctattgtcgcccttattagggcaagcggtgccagtagcagaatatgtcacctcagcaactcgatccgcccctgcccattacatgggtaacatatccatggaggttcgatgtatactcgaggatacagtcgcccatcacgccagcctacatacccattacatcagcatag

SEQ ID NO: 72 - DNA, 484 bp, Propionibacterium acnes
gttgcacaccagggggtcaacttggtgtcctcagttcaaaattgattcaaactaacggttccgtatcgggaaacagcaccagaaaactcgggacatatcgtctttcattgcgagaaaaatcttacttatgcgcatttctaagctatagcgtctacccttgccagacccaggacgatgagtgtcacatcccctttccagtcaacctaagagaggaggaaatgccgcgatatatgctccgccctgtcatcacgaaagccaccacaatctatcccagaacagccggcacttcactcacgatgccccgatgctggattcctattgtcgcccttattagggcaagcggtgccagtagcagaatatgtcacctcagcaactcgatccgcccctgcccattacatgggtaacatatccatggaggttcgatgtatactcgaggatacagtcgcccatcacgccagcctacatacccattacatcagcatag

SEQ ID NO: 73 - DNA, 484 bp, Propionibacterium acnes
gttgcacaccagggggtcaacttggtgtcctcagttcaaaattgattcaaactaacggttccgtatcgggaaacagcaccagaaaactcgggacatatcgtctttcattgcgagaaaaatcttacttatgcgcatttctaagctatatcgtctacccttgccagacccaggacgatgagtgtcacatcccctttccagtcaacctaagagaggaggaaatgccgcgatatatgctccgccctgtcatcacgaaagccaccacaatctatcccagaacagccggcacttcactcacgatgccccgatgctggattcctattgtcgcccttattagggcaagcggtgccagtagcagaatatgtcacctcagcaactcgatccgcccctgcccattacatgggtaacatatccatggaggttcgatgtatactcgaggatacagtcgcccatcacgccagcctacatacccattacatcagcatag

SEQ ID NO: 74 - DNA, 484 bp, Propionibacterium acnes
gttgcacaccagggggtcaacttggtgtcctcagttcaaaattgattcaaactaacggttccgtgtcgggaaacagcaccagaaaactcgggacatatcgtctttcattgcgagaaaaatcttacttatgcgcatttctaagctatagcgtctacccttgtcagacccaggacgatgagtgtcacatcccctttccagtcaacctaagagaggaggaaatgccgcgatatatgctccgccctgtcatcacgaaagccaccacaatctatcccagaacagccggcacttcactcacgatgccccgatgctggattcctattgtcgcccttattagggcaagcggtgccagtagcagaatatgtcacctcagcaactcgatccgcccctgcccattacatggttaacatatccatggaggttcgatgtatactcgaggatacagtcgcccatcacgccagcctacatacccattacatcagcatag

SEQ ID NO: 75 - DNA, 484 bp, Propionibacterium acnes
gttgcacaccagggggtcaacttggtgtcctcagttcaaaattgattcaaactaacggttccgtgtcgggaaacagcaccagaaaactcgggacatatcgtctttcattgcgagaaaaatcttacttatgcgcatttctaagctatagcgtctacccttgtcagacccaggacgatgagtgtcacatcccctttccagtcaacctaagagaggaggaaatgccgcgatatatgctccgccctgtcatcacgaaagccaccacaatctatcccagaacagccggcacttcactcacgatgccccgatgctggattcctattgtcgcccttattagggcaagcggtgccagtagcagaatatgtcacctcagcaactcgatccgcccctgcccattacatgggtaacatatccatggaggttcgatgtatactcgaggatacagtcgcccatcacgccagcctacatacccattacatcagcatag

SEQ ID NO: 76 - DNA, 484 bp, Propionibacterium acnes
gttgcacaccagggggtcaacttggtgtcctcagttcaaaattgattcaaactaacggttccgtatcgggaaacagcaccagaaaactcgggacatatcgtctttcattgcgagaaaaatcttacttatgcgcatttctaagctatagcgtctacccttgtcagacccaggacgatgagtgtcacatcccctttccagtcaacctaagagaggaggaaatgccgcgatatatgctccgccctgtcatcacgaaagccaccacaatctatcccagaacagccggcacttcactcacgatgccccgatgctggattcctattgtcgcccttattagggcaagcggtgccagtagcagaatatgtcacctcagcaactcgatccgcccccgcccattacatgggtaacatatccatggaggttcgatgtatactcgaggatacagtcgcccatcacgccagcctacatacccattacatcagcatag

SEQ ID NO: 77 - DNA, 21 bp, Artificial Sequence
  Synthetic Polynucleotide
cagcggcgctgctaagaactt

SEQ ID NO: 78 - DNA, 20 bp, Artificial Sequence
  Synthetic Polynucleotide
ccggctggcaaatgaggcat

SEQ ID NO: 79 - DNA, 54 bp, Artificial Sequence
  Synthetic Polynucleotide
tcgtcggcagcgtcagatgtgtataagagacagcagcggcgctgctaagaactt

SEQ ID NO: 80 - DNA, 54 bp, Artificial Sequence
  Synthetic Polynucleotide
gtctcgtgggctcggagatgtgtataagagacagccggctggcaaatgaggcat

SEQ ID NO: 81 - DNA, 54 bp, Artificial Sequence; identical to SEQ ID NO: 79
  Synthetic Polynucleotide

SEQ ID NO: 82 - DNA, 54 bp, Artificial Sequence; identical to SEQ ID NO: 80
  Synthetic Polynucleotide